European Patent Application EP 4 154 909 A1, published March 29, 2023. Title: DIAGNOSIS AND TREATMENT OF CANCERS SHOWING HIGH EXPRESSION OF PIWI AND/OR NMD COMPLEX PROTEIN. Applicant: SHANGHAITECH UNIVERSITY. The sequence listing filed with the application follows.

SEQUENCE LISTING (64 sequences)

SEQ ID NO: 1 - DNA, 20 bp, Artificial Sequence
  ACTB Forward Primer
ccctggagaagagctacgag

SEQ ID NO: 2 - DNA, 20 bp, Artificial Sequence
  ACTB Reverse Primer
ggaaggaaggctggaagagt

SEQ ID NO: 3 - DNA, 20 bp, Artificial Sequence
  PIWIL1 Forward Primer
cagccaagtcacaaggactc

SEQ ID NO: 4 - DNA, 20 bp, Artificial Sequence
  PIWIL1 Reverse Primer
gatgtcagccggaaatggtt

SEQ ID NO: 5 - DNA, 20 bp, Artificial Sequence
  PIWIL2 Forward Primer
ttggttggagtaggacgctt

SEQ ID NO: 6 - DNA, 20 bp, Artificial Sequence
  PIWIL2 Reverse Primer
aaggtacagggaggcttgtc

SEQ ID NO: 7 - DNA, 20 bp, Artificial Sequence
  PIWIL4 Forward Primer
gatggcaccgagatcaccta

SEQ ID NO: 8 - DNA, 20 bp, Artificial Sequence
  PIWIL4 Reverse Primer
tggtcagtcagccctgttag

SEQ ID NO: 9 - DNA, 20 bp, Artificial Sequence
  UPF1 Forward Primer
atccgcctgcaggtccagta

SEQ ID NO: 10 - DNA, 20 bp, Artificial Sequence
  UPF1 Reverse Primer
gatccgctgcagtgacacca

SEQ ID NO: 11 - DNA, 20 bp, Artificial Sequence
  FLNA Forward Primer
gggatcccatccctaagagc

SEQ ID NO: 12 - DNA, 20 bp, Artificial Sequence
  FLNA Reverse Primer
cttggatgccactttgcctt

SEQ ID NO: 13 - DNA, 20 bp, Artificial Sequence
  LAMC3 Forward Primer
actgtgagcactgtcaggaa

SEQ ID NO: 14 - DNA, 20 bp, Artificial Sequence
  LAMC3 Reverse Primer
tgcaaggcatgcatttgtct

SEQ ID NO: 15 - DNA, 20 bp, Artificial Sequence
  CCNE2
gggggatcagtccttgcatt

SEQ ID NO: 16 - DNA, 20 bp, Artificial Sequence
  CCNE2 Reverse Primer
aaggcagcagcagtcagtat

SEQ ID NO: 17 - DNA, 20 bp, Artificial Sequence
  ORC6 Forward Primer
atgctgaggaaagcagagga

SEQ ID NO: 18 - DNA, 20 bp, Artificial Sequence
  ORC6 Reverse Primer
ttcatccaggaagctgcaag

SEQ ID NO: 19 - DNA, 20 bp, Artificial Sequence
  CDC25A Forward Primer
gtgccggtatgtgagagaga

SEQ ID NO: 20 - DNA, 20 bp, Artificial Sequence
  CDC25A Reverse Primer
tgcggaacttcttcaggtct

SEQ ID NO: 21 - DNA, 20 bp, Artificial Sequence
  MCM2 Forward Primer
cgagatagagctgactggca

SEQ ID NO: 22 - DNA, 20 bp, Artificial Sequence
  MCM2 Reverse Primer
cagtggcaaagacagggaag

SEQ ID NO: 23 - DNA, 20 bp, Artificial Sequence
  CCND3 Forward Primer
atcactggcactgaagtgga

SEQ ID NO: 24 - DNA, 20 bp, Artificial Sequence
  CCND3 Reverse Primer
tctgtaggagtgctggtctg

SEQ ID NO: 25 - DNA, 20 bp, Artificial Sequence
  PCNA Forward Primer
gcgtgaacctcaccagtatg

SEQ ID NO: 26 - DNA, 20 bp, Artificial Sequence
  PCNA Reverse Primer
tctcctggtttggtgcttca

SEQ ID NO: 27 - DNA, 20 bp, Artificial Sequence
  MYO18B Forward Primer
gaagcagatgcaccagaagg

SEQ ID NO: 28 - DNA, 20 bp, Artificial Sequence
  MYO18B Reverse Primer
ccaatctggtcacagagggt

SEQ ID NO: 29 - DNA, 20 bp, Artificial Sequence
  VCL Forward Primer
gaccggccaaagcagctgta

SEQ ID NO: 30 - DNA, 20 bp, Artificial Sequence
  VCL Reverse Primer
gatggcagcctgaccgactc

SEQ ID NO: 31 - DNA, 20 bp, Artificial Sequence
  SESN2
ggctggaggcactgatgtcc

SEQ ID NO: 32 - DNA, 20 bp, Artificial Sequence
  SESN2 Reverse Primer
tagtcagggtgcaggcccat

SEQ ID NO: 33 - DNA, 20 bp, Artificial Sequence
  SRCIN1 Forward Primer
acagagctcaaggctcactt

SEQ ID NO: 34 - DNA, 20 bp, Artificial Sequence
  SRCIN1 Reverse Primer
ggctcctccttcaggaactt

SEQ ID NO: 35 - DNA, 20 bp, Artificial Sequence
  TPM2 Forward Primer
gatgctgaagctggacaagg

SEQ ID NO: 36 - DNA, 20 bp, Artificial Sequence
  TPM2 Reverse Primer
ggtcctcagcttgcttcttg

SEQ ID NO: 37 - DNA, 20 bp, Artificial Sequence
  DDIT4 Forward Primer
gagtccctggacagcagcaa

SEQ ID NO: 38 - DNA, 20 bp, Artificial Sequence
  DDIT4 Reverse Primer
cagcagctgcatcaggttgg

SEQ ID NO: 39 - DNA, 20 bp, Artificial Sequence
  CCDC80Forward Primer
agcagaagaaggagggcatt

SEQ ID NO: 40 - DNA, 20 bp, Artificial Sequence
  CCDC80 Reverse Primer
agatcaccagcaacctcctc

SEQ ID NO: 41 - DNA, 20 bp, Artificial Sequence
  PTEN Forward Primer
gcggaacttgcaatcctcag

SEQ ID NO: 42 - DNA, 20 bp, Artificial Sequence
  PTEN Reverse Primer
gaacttgtcttcccgtcgtg

SEQ ID NO: 43 - DNA, 20 bp, Artificial Sequence
  GADD45G Forward Primer
agctgctggttgatcgcact

SEQ ID NO: 44 - DNA, 20 bp, Artificial Sequence
  GADD45G Reverse Primer
agcaactcatgcagcgcttt

SEQ ID NO: 45 - DNA, 20 bp, Artificial Sequence
  GADD45B Forward Primer
tgaatgtggacccagacagc

SEQ ID NO: 46 - DNA, 20 bp, Artificial Sequence
  GADD45B Reverse Primer
aaggactggatgagcgtgaa

SEQ ID NO: 47 - DNA, 20 bp, Artificial Sequence
  TSC2 Forward Primer
tactgcgtctgcgactacat

SEQ ID NO: 48 - DNA, 20 bp, Artificial Sequence
  TSC2 Reverse Primer
ccagtcagactcctgcttca

SEQ ID NO: 49 - DNA, 20 bp, Artificial Sequence
  TP53 Forward Primer
gtccagatgaagctcccaga

SEQ ID NO: 50 - DNA, 20 bp, Artificial Sequence
  TP53 Reverse Primer
caagaagcccagacggaaac

SEQ ID NO: 51 - DNA, 20 bp, Artificial Sequence
  MCM10 Forward Primer
gtggaagccttctctggtct

SEQ ID NO: 52 - DNA, 20 bp, Artificial Sequence
  MCM10 Reverse Primer
cagcttctctctggccatct

SEQ ID NO: 53 - DNA, 57 bp, Artificial Sequence
  2U6 hPiwil-1 E5 sg2 Forward Primer
atgcgtctcaaccgcattgactataacccactgagttttagagctagaaatagcaag

SEQ ID NO: 54 - DNA, 57 bp, Artificial Sequence
  2U6 hPiwil-1 E5 sg1 Reverse Primer
atgcgtctcgaaacgctgacatcccgtccccagtcggtgtttcgtcctttccacaag

SEQ ID NO: 55 - DNA, 19 bp, Artificial Sequence
  hPiwil-1 E5 C9 (genomePCR) Forward Primer
actgtgcctgccttgtcat

SEQ ID NO: 56 - DNA, 23 bp, Artificial Sequence
  hPiwil-1 E5 C9 (genomePCR) Reverse Primer
ggtagttctgctttgaagtggaa

SEQ ID NO: 57 - DNA, 115 bp, Artificial Sequence
  PIWIL1-piRNA-binding mutant Forward Primer
gcaaaatacctgtgtacagattgccctaccccaagtgcatgtgtggtggcccgaaccttaggcaaacagcaaactgtcatggccattgctacaaagattgccctagcaatgaact

SEQ ID NO: 58 - DNA, 30 bp, Artificial Sequence
  PIWIL1-piRNA-binding mutant Reverse Primer
aatagcatcgtatttgtccttccgattact

SEQ ID NO: 59 - DNA, 39 bp, Artificial Sequence
  (2-250)/(2-624)-Forward Primer
gatgatgacgacaaaggatccactgggagagcccgagcc

SEQ ID NO: 60 - DNA, 26 bp, Artificial Sequence
  (2-250)-Reverse Primer
tcaggaggccaaatcaccaacctgtg

SEQ ID NO: 61 - DNA, 40 bp, Artificial Sequence
  (384-861)/(384-624)-Forward Primer
ttggtgatttggcctcctgagctctgctatcttacaggtc

SEQ ID NO: 62 - DNA, 45 bp, Artificial Sequence
  (384-861)/(759-861)-Reverse Primer
aacgggccctctagactcgagttagaggtagtaaaggcggtttga

SEQ ID NO: 63 - DNA, 35 bp, Artificial Sequence
  (2-624)/(384-624)-Reverse Primer
tgttccaggaagtggcttcagggggatgtccaccc

SEQ ID NO: 64 - DNA, 30 bp, Artificial Sequence
  (759-861)-Forward Primer
tgaagccacttcctggaacagttattgatg